European Patent Specification EP 3 328 898 B1, published March 6, 2024. Title: TRKB OR TRKC AGONIST COMPOSITIONS AND METHODS FOR THE TREATMENT OF OTIC CONDITIONS. Applicant: OTONOMY, INC. The sequence listing filed with the application follows.

SEQUENCE LISTING (120 sequences)

SEQ ID NO: 1 - protein, 18 aa, Artificial Sequence
  Description of Artificial Sequence: Synthetic peptide
ESTDNFILFDEVSPTPPI

SEQ ID NO: 2 - protein, 10 aa, Artificial Sequence
  Description of Artificial Sequence: Synthetic peptide
  MOD_RES (8)..(8): R or W
  MOD_RES (9)..(9): I, L, R, or M
GYTFTSYXXH

SEQ ID NO: 3 - protein, 17 aa, Artificial Sequence
  Description of Artificial Sequence: Synthetic peptide
  MOD_RES (7)..(7): A, T, S, or G
  MOD_RES (16)..(16): K or E
EIYPSNXRTNYNEKFXS

SEQ ID NO: 4 - protein, 15 aa, Artificial Sequence
  Description of Artificial Sequence: Synthetic peptide
  MOD_RES (7)..(7): T or S
  MOD_RES (8)..(8): R, Q, K, S, or Y
KYYYGNXXRSWYFDV

SEQ ID NO: 5 - protein, 10 aa, Artificial Sequence
  Description of Artificial Sequence: Synthetic peptide
GYTFTSYWMH

SEQ ID NO: 6 - protein, 16 aa, Artificial Sequence
  Description of Artificial Sequence: Synthetic peptide
EIYPSNGRTNYNEKFK

SEQ ID NO: 7 - protein, 15 aa, Artificial Sequence
  Description of Artificial Sequence: Synthetic peptide
KYYYGNSYRSWYFDV

SEQ ID NO: 8 - protein, 17 aa, Artificial Sequence
  Description of Artificial Sequence: Synthetic peptide
KSSQSVSYSSNNKNYLA

SEQ ID NO: 9 - protein, 7 aa, Artificial Sequence
  Description of Artificial Sequence: Synthetic peptide
WASTRES

SEQ ID NO: 10 - protein, 9 aa, Artificial Sequence
  Description of Artificial Sequence: Synthetic peptide
QQHYNTPLT

SEQ ID NO: 11 - protein, 7 aa, Artificial Sequence
  Description of Artificial Sequence: Synthetic peptide
ISTYYWN

SEQ ID NO: 12 - protein, 16 aa, Artificial Sequence
  Description of Artificial Sequence: Synthetic peptide
RIYTSGSTNYNPSLKS

SEQ ID NO: 13 - protein, 9 aa, Artificial Sequence
  Description of Artificial Sequence: Synthetic peptide
DGGYSNPFD

SEQ ID NO: 14 - protein, 11 aa, Artificial Sequence
  Description of Artificial Sequence: Synthetic peptide
RTSENVYSNLA

SEQ ID NO: 15 - protein, 7 aa, Artificial Sequence
  Description of Artificial Sequence: Synthetic peptide
AASNLQS

SEQ ID NO: 16 - protein, 9 aa, Artificial Sequence
  Description of Artificial Sequence: Synthetic peptide
QHFWGSPFT

SEQ ID NO: 17 - protein, 5 aa, Artificial Sequence
  Description of Artificial Sequence: Synthetic peptide
NYDII

SEQ ID NO: 18 - protein, 6 aa, Artificial Sequence
  Description of Artificial Sequence: Synthetic peptide
PYNDGT

SEQ ID NO: 19 - protein, 14 aa, Artificial Sequence
  Description of Artificial Sequence: Synthetic peptide
LLKYRRFRYYAIDY

SEQ ID NO: 20 - protein, 11 aa, Artificial Sequence
  Description of Artificial Sequence: Synthetic peptide
RASQTISNNLH

SEQ ID NO: 21 - protein, 7 aa, Artificial Sequence
  Description of Artificial Sequence: Synthetic peptide
SASLAIS

SEQ ID NO: 22 - protein, 9 aa, Artificial Sequence
  Description of Artificial Sequence: Synthetic peptide
QQSNSWPNT

SEQ ID NO: 23 - protein, 10 aa, Artificial Sequence
  Description of Artificial Sequence: Synthetic peptide
GYSFTAYFMN

SEQ ID NO: 24 - protein, 17 aa, Artificial Sequence
  Description of Artificial Sequence: Synthetic peptide
RINPNNGDTFYTQKFKG

SEQ ID NO: 25 - protein, 9 aa, Artificial Sequence
  Description of Artificial Sequence: Synthetic peptide
RDYFGAMDY

SEQ ID NO: 26 - protein, 16 aa, Artificial Sequence
  Description of Artificial Sequence: Synthetic peptide
RSSQSLVHSNGNTYLH

SEQ ID NO: 27 - protein, 7 aa, Artificial Sequence
  Description of Artificial Sequence: Synthetic peptide
KVSNRFS

SEQ ID NO: 28 - protein, 9 aa, Artificial Sequence
  Description of Artificial Sequence: Synthetic peptide
SQGTHVPYT

SEQ ID NO: 29 - protein, 5 aa, Artificial Sequence
  Description of Artificial Sequence: Synthetic peptide
DYEMH

SEQ ID NO: 30 - protein, 17 aa, Artificial Sequence
  Description of Artificial Sequence: Synthetic peptide
TIDPETAGTAYNQKFKG

SEQ ID NO: 31 - protein, 7 aa, Artificial Sequence
  Description of Artificial Sequence: Synthetic peptide
VTTWFAY

SEQ ID NO: 32 - protein, 16 aa, Artificial Sequence
  Description of Artificial Sequence: Synthetic peptide
RSSQSLIHSNGNTYLH

SEQ ID NO: 33 - protein, 7 aa, Artificial Sequence
  Description of Artificial Sequence: Synthetic peptide
KVSNRFS

SEQ ID NO: 34 - protein, 9 aa, Artificial Sequence
  Description of Artificial Sequence: Synthetic peptide
SQSTHVPFT

SEQ ID NO: 35 - protein, 5 aa, Artificial Sequence
  Description of Artificial Sequence: Synthetic peptide
SYDIN

SEQ ID NO: 36 - protein, 17 aa, Artificial Sequence
  Description of Artificial Sequence: Synthetic peptide
WIYPRDGSIKFNEKFKG

SEQ ID NO: 37 - protein, 11 aa, Artificial Sequence
  Description of Artificial Sequence: Synthetic peptide
RGRLLLYGFAY

SEQ ID NO: 38 - protein, 15 aa, Artificial Sequence
  Description of Artificial Sequence: Synthetic peptide
RASKSVSTSGYSYMH

SEQ ID NO: 39 - protein, 7 aa, Artificial Sequence
  Description of Artificial Sequence: Synthetic peptide
LVSNLES

SEQ ID NO: 40 - protein, 9 aa, Artificial Sequence
  Description of Artificial Sequence: Synthetic peptide
QHIRELTRS

SEQ ID NO: 41 - protein, 7 aa, Artificial Sequence
  Description of Artificial Sequence: Synthetic peptide
FWIEWVK

SEQ ID NO: 42 - protein, 17 aa, Artificial Sequence
  Description of Artificial Sequence: Synthetic peptide
EILPGSDNTNYNEKFKG

SEQ ID NO: 43 - protein, 11 aa, Artificial Sequence
  Description of Artificial Sequence: Synthetic peptide
KNRNYYGNYVV

SEQ ID NO: 44 - protein, 10 aa, Artificial Sequence
  Description of Artificial Sequence: Synthetic peptide
SASSSVSYMY

SEQ ID NO: 45 - protein, 7 aa, Artificial Sequence
  Description of Artificial Sequence: Synthetic peptide
STSNLAS

SEQ ID NO: 46 - protein, 9 aa, Artificial Sequence
  Description of Artificial Sequence: Synthetic peptide
QQRSSYPLT

SEQ ID NO: 47 - protein, 7 aa, Artificial Sequence
  Description of Artificial Sequence: Synthetic peptide
FWIEWVK

SEQ ID NO: 48 - protein, 17 aa, Artificial Sequence
  Description of Artificial Sequence: Synthetic peptide
EILPGSDNTNYNEKFKG

SEQ ID NO: 49 - protein, 11 aa, Artificial Sequence
  Description of Artificial Sequence: Synthetic peptide
KNRNYYGNYVV

SEQ ID NO: 50 - protein, 16 aa, Artificial Sequence
  Description of Artificial Sequence: Synthetic peptide
  MOD_RES (7)..(7): V or I
  MOD_RES (9)..(9): N or S
  MOD_RES (15)..(15): M or L
  MOD_RES (16)..(16): N, T or A
RASESVXDXYGISFXX

SEQ ID NO: 51 - protein, 7 aa, Artificial Sequence
  Description of Artificial Sequence: Synthetic peptide
  MOD_RES (5)..(5): Q, L or R
AASNXGS

SEQ ID NO: 52 - protein, 9 aa, Artificial Sequence
  Description of Artificial Sequence: Synthetic peptide
  MOD_RES (5)..(5): E or T
QQSKXVPRT

SEQ ID NO: 53 - protein, 7 aa, Artificial Sequence
  Description of Artificial Sequence: Synthetic peptide
  MOD_RES (2)..(2): W or M
  MOD_RES (3)..(3): M, I or L
YXXHWVK

SEQ ID NO: 54 - protein, 17 aa, Artificial Sequence
  Description of Artificial Sequence: Synthetic peptide
  MOD_RES (7)..(7): G, S, A or T
  MOD_RES (16)..(16): K or E
EIYPSNXRTNYNEKFXS

SEQ ID NO: 55 - protein, 15 aa, Artificial Sequence
  Description of Artificial Sequence: Synthetic peptide
  MOD_RES (7)..(7): S or T
  MOD_RES (8)..(8): Y or R
KYYYGNXXRSWYFDV

SEQ ID NO: 56 - protein, 12 aa, Artificial Sequence
  Description of Artificial Sequence: Synthetic peptide
RASQSVSSNYLT

SEQ ID NO: 57 - protein, 7 aa, Artificial Sequence
  Description of Artificial Sequence: Synthetic peptide
GASSRAT

SEQ ID NO: 58 - protein, 10 aa, Artificial Sequence
  Description of Artificial Sequence: Synthetic peptide
QQYGRSPPIT

SEQ ID NO: 59 - protein, 7 aa, Artificial Sequence
  Description of Artificial Sequence: Synthetic peptide
SGGYYWS

SEQ ID NO: 60 - protein, 16 aa, Artificial Sequence
  Description of Artificial Sequence: Synthetic peptide
YIFYSGRTYYNPSLKS

SEQ ID NO: 61 - protein, 17 aa, Artificial Sequence
  Description of Artificial Sequence: Synthetic peptide
ERIAAAGADYYYNGLDV

SEQ ID NO: 62 - protein, 12 aa, Artificial Sequence
  Description of Artificial Sequence: Synthetic peptide
RASQSGSSTYLA

SEQ ID NO: 63 - protein, 7 aa, Artificial Sequence
  Description of Artificial Sequence: Synthetic peptide
GASSRAT

SEQ ID NO: 64 - protein, 10 aa, Artificial Sequence
  Description of Artificial Sequence: Synthetic peptide
QQYGRSPPIT

SEQ ID NO: 65 - protein, 7 aa, Artificial Sequence
  Description of Artificial Sequence: Synthetic peptide
SGYYYWS

SEQ ID NO: 66 - protein, 16 aa, Artificial Sequence
  Description of Artificial Sequence: Synthetic peptide
YIYYSGSTYYNPSLKS

SEQ ID NO: 67 - protein, 17 aa, Artificial Sequence
  Description of Artificial Sequence: Synthetic peptide
ERIAAAGTDYYYNGLAV

SEQ ID NO: 68 - protein, 11 aa, Artificial Sequence
  Description of Artificial Sequence: Synthetic peptide
RASQGIRNDLG

SEQ ID NO: 69 - protein, 7 aa, Artificial Sequence
  Description of Artificial Sequence: Synthetic peptide
AASSLQS

SEQ ID NO: 70 - protein, 9 aa, Artificial Sequence
  Description of Artificial Sequence: Synthetic peptide
LQHNSLPLT

SEQ ID NO: 71 - protein, 7 aa, Artificial Sequence
  Description of Artificial Sequence: Synthetic peptide
SGGYYWS

SEQ ID NO: 72 - protein, 16 aa, Artificial Sequence
  Description of Artificial Sequence: Synthetic peptide
YIYYSGSTNYNPSLKS

SEQ ID NO: 73 - protein, 18 aa, Artificial Sequence
  Description of Artificial Sequence: Synthetic peptide
DRDYDSTGDYYSYYGMDV

SEQ ID NO: 74 - protein, 11 aa, Artificial Sequence
  Description of Artificial Sequence: Synthetic peptide
RASENVYSNLA

SEQ ID NO: 75 - protein, 7 aa, Artificial Sequence
  Description of Artificial Sequence: Synthetic peptide
AASNLQS

SEQ ID NO: 76 - protein, 9 aa, Artificial Sequence
  Description of Artificial Sequence: Synthetic peptide
QHFWGSPFT

SEQ ID NO: 77 - protein, 10 aa, Artificial Sequence
  Description of Artificial Sequence: Synthetic peptide
GYTFTNYDII

SEQ ID NO: 78 - protein, 15 aa, Artificial Sequence
  Description of Artificial Sequence: Synthetic peptide
YINPYNRRREYNEKF

SEQ ID NO: 79 - protein, 14 aa, Artificial Sequence
  Description of Artificial Sequence: Synthetic peptide
LLKYRRFRYYAIDY

SEQ ID NO: 80 - protein, 11 aa, Artificial Sequence
  Description of Artificial Sequence: Synthetic peptide
RASENVYSNLA

SEQ ID NO: 81 - protein, 7 aa, Artificial Sequence
  Description of Artificial Sequence: Synthetic peptide
AASNLAD

SEQ ID NO: 82 - protein, 9 aa, Artificial Sequence
  Description of Artificial Sequence: Synthetic peptide
QHFWYSPFT

SEQ ID NO: 83 - protein, 5 aa, Artificial Sequence
  Description of Artificial Sequence: Synthetic peptide
NYDII

SEQ ID NO: 84 - protein, 6 aa, Artificial Sequence
  Description of Artificial Sequence: Synthetic peptide
PYNDGT

SEQ ID NO: 85 - protein, 14 aa, Artificial Sequence
  Description of Artificial Sequence: Synthetic peptide
LLKYRRFSYYAIDY

SEQ ID NO: 86 - protein, 11 aa, Artificial Sequence
  Description of Artificial Sequence: Synthetic peptide
RASENVYSNLA

SEQ ID NO: 87 - protein, 7 aa, Artificial Sequence
  Description of Artificial Sequence: Synthetic peptide
AASNLQS

SEQ ID NO: 88 - protein, 9 aa, Artificial Sequence
  Description of Artificial Sequence: Synthetic peptide
QHFWYSPWT

SEQ ID NO: 89 - protein, 5 aa, Artificial Sequence
  Description of Artificial Sequence: Synthetic peptide
NYDII

SEQ ID NO: 90 - protein, 6 aa, Artificial Sequence
  Description of Artificial Sequence: Synthetic peptide
PYNDGT

SEQ ID NO: 91 - protein, 14 aa, Artificial Sequence
  Description of Artificial Sequence: Synthetic peptide
LLKYRRFRYYAIDY

SEQ ID NO: 92 - protein, 11 aa, Artificial Sequence
  Description of Artificial Sequence: Synthetic peptide
HASENVYSNLA

SEQ ID NO: 93 - protein, 7 aa, Artificial Sequence
  Description of Artificial Sequence: Synthetic peptide
AASNLQS

SEQ ID NO: 94 - protein, 9 aa, Artificial Sequence
  Description of Artificial Sequence: Synthetic peptide
QHFWGSPFT

SEQ ID NO: 95 - protein, 5 aa, Artificial Sequence
  Description of Artificial Sequence: Synthetic peptide
NYDII

SEQ ID NO: 96 - protein, 6 aa, Artificial Sequence
  Description of Artificial Sequence: Synthetic peptide
PYNRRR

SEQ ID NO: 97 - protein, 14 aa, Artificial Sequence
  Description of Artificial Sequence: Synthetic peptide
LLKYRRFRYYAIDY

SEQ ID NO: 98 - protein, 11 aa, Artificial Sequence
  Description of Artificial Sequence: Synthetic peptide
RASEPVYSNVA

SEQ ID NO: 99 - protein, 7 aa, Artificial Sequence
  Description of Artificial Sequence: Synthetic peptide
AASNLQS

SEQ ID NO: 100 - protein, 9 aa, Artificial Sequence
  Description of Artificial Sequence: Synthetic peptide
QHFWGSPFT

SEQ ID NO: 101 - protein, 5 aa, Artificial Sequence
  Description of Artificial Sequence: Synthetic peptide
NYDII

SEQ ID NO: 102 - protein, 6 aa, Artificial Sequence
  Description of Artificial Sequence: Synthetic peptide
PYNGRR

SEQ ID NO: 103 - protein, 14 aa, Artificial Sequence
  Description of Artificial Sequence: Synthetic peptide
LLKYRRFRYYAIDY

SEQ ID NO: 104 - protein, 5 aa, Artificial Sequence
  Description of Artificial Sequence: Synthetic peptide
AYFMN

SEQ ID NO: 105 - protein, 13 aa, Artificial Sequence
  Description of Artificial Sequence: Synthetic peptide
CSLSSQHSTYTIE

SEQ ID NO: 106 - protein, 7 aa, Artificial Sequence
  Description of Artificial Sequence: Synthetic peptide
LKKDGSH

SEQ ID NO: 107 - protein, 14 aa, Artificial Sequence
  Description of Artificial Sequence: Synthetic peptide
CGVGDTIKEQFVYV

SEQ ID NO: 108 - protein, 11 aa, Artificial Sequence
  Description of Artificial Sequence: Synthetic peptide
SGFNIKDTYMH

SEQ ID NO: 109 - protein, 17 aa, Artificial Sequence
  Description of Artificial Sequence: Synthetic peptide
IDPAHNNIKYDPKFQGK

SEQ ID NO: 110 - protein, 11 aa, Artificial Sequence
  Description of Artificial Sequence: Synthetic peptide
CTGSLGRGDYF

SEQ ID NO: 111 - protein, 15 aa, Artificial Sequence
  Description of Artificial Sequence: Synthetic peptide
CRSSTGAVTTSNYAS

SEQ ID NO: 112 - protein, 7 aa, Artificial Sequence
  Description of Artificial Sequence: Synthetic peptide
GGTNNRA

SEQ ID NO: 113 - protein, 10 aa, Artificial Sequence
  Description of Artificial Sequence: Synthetic peptide
CALCYSNHLV

SEQ ID NO: 114 - protein, 11 aa, Artificial Sequence
  Description of Artificial Sequence: Synthetic peptide
SGFTFSNYAMS

SEQ ID NO: 115 - protein, 16 aa, Artificial Sequence
  Description of Artificial Sequence: Synthetic peptide
ISSGGSTYYPDSVKGR

SEQ ID NO: 116 - protein, 18 aa, Artificial Sequence
  Description of Artificial Sequence: Synthetic peptide
CARGRGLRLRSYYYALDY

SEQ ID NO: 117 - protein, 119 aa, Unknown [sequence omitted]

SEQ ID NO: 118 - protein, 20 aa, Artificial Sequence
  Description of Artificial Sequence: Synthetic peptide
TITFLESPTSDHHWCIPFTV

SEQ ID NO: 119 - protein, 6 aa, Unknown
  Description of Unknown: Neurotrophin-3 peptide
YAEHKS

SEQ ID NO: 120 - protein, 7 aa, Unknown
  Description of Unknown: Neurotrophin-3 peptide
SSSHPIF